European Patent Application EP 4 471 426 A2, published December 4, 2024. Title: Method and reagents for the detection of a mammalian antibody. Applicant: EUROIMMUN Medizinische Labordiagnostika AG. Application EP. The sequence listing filed with the application follows.

SEQUENCE LISTING (57 sequences)

SEQ ID NO: 1 - protein, 50 aa, synthetic construct
  source 1..50: note = fragment of ZSCAN5ABC
ESDPIQALRKLTELCHLWLRPDLHTKEQILDMLVMEQFMISMPQELQVLV

SEQ ID NO: 2 - protein, 23 aa, synthetic construct
  source 1..23: note = fragment of ZSCAN5ABC
NGVQSCKDLEDLLRNNRRPKKWS

SEQ ID NO: 3 - protein, 20 aa, synthetic construct
  source 1..20: note = fragment of ZSCAN5ABC
ASVENVDADTPSACVVEREA

SEQ ID NO: 4 - protein, 23 aa, synthetic construct
  source 1..23: note = fragment of ZSCAN5ABC
SISQEEPQGEATPVGNRESPGQA

SEQ ID NO: 5 - protein, 496 aa, Homo sapiens
  source 1..496: note = ZSCAN5A
MAANCTSSWSLGESCNRPGLELPRSMASSETQLGNHDVDPEISHVNFRMFSCPKESDPIQALRKLTELCHLWLRPDLHTKEQILDMLVMEQFMISMPQELQVLVMMNGVQSCKDLEDLLRNNRRPKKWSVVTFHGKEYIVQDSDIEMAEAPSSVRDDLKDVSSQRASSVNQMRPGEGQAHRELQILPRVPALSRRQGEDFLLHKSIDVTGDPKSLRPKQTLEKDLKENREENPGLTSPEPQLPKSPTDLVRAKEGKDPPKIASVENVDADTPSACVVEREASTHSGNRGDALNLSSPKRSKPDASSISQEEPQGEATPVGNRESPGQAGMNSIHSPGPASPVSHPDGQEAKALPPFACDVCEKRFTCNSKLVIHKRSHTGERLFQCNLCGKRFMQLISLQFHQRTHTGERPYTCDVCQKQFTQKSYLKCHKRSHTGEKPFECKDCKKVFTYRGSLKEHQRIHSGEKPYKCSKCPRAFSRLKLLRRHQKTHPEATSQ

SEQ ID NO: 6 - protein, 495 aa, Homo sapiens
  source 1..495: note = ZSCAN5B
MAANWTLSWGQGGPCNSPGSDTPRSVASPETQLGNHDRNPETWHMNFRMFSCPEESDPIQALRKLTELCHLWLRPDLHTKEQILDMLVMEQFMISMPQELQVLVKVNGVQSCKDLEDLLRNNRRPKKWSIVNLLGKEYLMLNSDVEMAEAPASVRDDPRDVSSQWASSVNQMHPGTGQARREQQILPRVAALSRRQGEDFLLHKSIDVTGDPNSPRPKQTLEKDLKENREENPGLSSPEPQLPKSPNLVRAKEGKEPQKRASVENVDADTPSACVVEREALTHSGNRGDALNLSSPKRSKPDASSISQEEPQGEATPVGNRESPGQAEINPVHSPGPAGPVSHPDGQEAKALPPFACDVCNKSFKYFSQLSIHRRSHTGDRPFQCDLCRKRFLQPSDLRVHQRVHTGERPYMCDVCQKRFAHESTLQGHKRIHTGERPFKCKYCSKVFSHKGNLNVHQRTHSGEKPYKCPTCQKAFRQLGTFKRHLKTHRETTSQ

SEQ ID NO: 7 - protein, 496 aa, Homo sapiens
  source 1..496: note = ZSCAN5C
MAANCTSSWSLGESCNSPGSEPPQSMPSPATQLGNHDSDPETCHVNFRMFSCPKESDPIQALRKLTELCHLWLRPDLHTKEQILDMLVMEQFMISMPQELQVLVMMNGVQSCKDLEDLLRNNRRPKKWSVVSFLGKEYLMQESDVEMAEAPASVRDDPRHVSSQRTSSVNQMCPEEGQASQELQTLPRVPALFRRQEEDFLLPETTVMKGDPKALRPKPTLEKDLEEDREENPGLTSPEPQLPNSPTGVVGAKEGKEPQKRASVENVDADTPSACVVEREASTHSGSRGDALNLRGLKRSKPDATSISQEEPQGEATPVGNRESPGQAEINPVHSPGPAGPVSHPSGQEVKELLPFACEVCGKRFKYRGKLAVHTRSHTGERLFQCNLCGKRFMQRIGLQFHQRTHTGERPYTCDICQKQFTQKSYLKCHKRSHTGEKPFECKDCKKVFTYKANLKEHQRIHSGEKPHKCSKCPRAFGRPATLRRHQKTHREATSQ

SEQ ID NO: 8 - protein, 91 aa, synthetic construct
  SITE 1: note = T or absent
  SITE 2: note = P or absent
  SITE 12: note = S or L
  SITE 17: note = S or N
  SITE 25: note = S or R
  SITE 26: note = S or G
  SITE 27: note = P or L
  SITE 35: note = S or T
  SITE 59: note = G or E
  SITE 60: note = M or I
  SITE 62: note = S or P
  SITE 63: note = I or V
  SITE 70: note = S or G
  SITE 76: note = D or S
  SITE 80: note = A or V
  SITE 82: note = A or E
  SITE 84: note = P or L
  SITE 89: note = D or E
  SITE 91: note = C or absent
XXSACVVEREAXTHSGXRGDALNLXXXKRSKPDAXSISQEEPQGEATPVGNRESPGQAXXNXXHSPGPAXPVSHPXGQEXKXLXPFACXVX

SEQ ID NO: 9 - protein, 16 aa, synthetic construct
MAANCTSSWSLGESCN

SEQ ID NO: 10 - protein, 88 aa, synthetic construct
HVNFRMFSCPKESDPIQALRKLTELCHLWLRPDLHTKEQILDMLVMEQFMISMPQELQVLVMMNGVQSCKDLEDLLRNNRRPKKWSVV

SEQ ID NO: 11 - protein, 15 aa, synthetic construct
REENPGLTSPEPQLP

SEQ ID NO: 12 - protein, 25 aa, synthetic construct
ASVENVDADTPSACVVEREASTHSG

SEQ ID NO: 13 - protein, 20 aa, synthetic construct
RSHTGERLFQCNLCGKRFMQ

SEQ ID NO: 14 - protein, 17 aa, synthetic construct
LQFHQRTHTGERPYTCD

SEQ ID NO: 15 - protein, 35 aa, synthetic construct
CQKQFTQKSYLKCHKRSHTGEKPFECKDCKKVFTY

SEQ ID NO: 16 - protein, 13 aa, synthetic construct
LKEHQRIHSGEKP

SEQ ID NO: 17 - protein, 9 aa, synthetic construct
KCSKCPRAF

SEQ ID NO: 18 - protein, 17 aa, synthetic construct
SDVEMAEAPASVRDDPR

SEQ ID NO: 19 - protein, 30 aa, synthetic construct
AKEGKEPQKRASVENVDADTPSACVVEREA

SEQ ID NO: 20 - protein, 40 aa, synthetic construct
SISQEEPQGEATPVGNRESPGQAEINPVHSPGPAGPVSHP

SEQ ID NO: 21 - protein, 22 aa, synthetic construct
ALSRRQGEDFLLHKSIDVTGDP

SEQ ID NO: 22 - protein, 20 aa, synthetic construct
RPKQTLEKDLKENREENPGL

SEQ ID NO: 23 - protein, 46 aa, synthetic construct
THSGNRGDALNLSSPKRSKPDASSISQEEPQGEATPVGNRESPGQA

SEQ ID NO: 24 - protein, 21 aa, synthetic construct
PVSHPDGQEAKALPPFACDVC

SEQ ID NO: 25 - DNA, 747 bp, synthetic construct
  source 1..747: mol_type = other DNA; note = ZSCAN5B, gene synthesis fragment 1, coding aa1-242
atacgtctcacatggctgcaaattggacactctcatggggtcagggaggaccctgcaacagccctgggtcagacactccacggtctgtggcgtccccagaaactcaacttggaaatcacgacaggaaccctgagacttggcacatgaatttcaggatgttcagctgcccagaggagtcggaccccatccaggctctgaggaaactcactgagctgtgccatctgtggctgaggcccgacctccacaccaaagagcagatcctggacatgctggtgatggagcagttcatgatctccatgccccaggagctccaggtcttagtcaaggtgaacggtgtgcagagctgcaaagacctggaggacctgctacgaaataacagaagacccaagaaatggtctatagtcaacttgctcggcaaagaatatcttatgctgaactcagatgtcgagatggctgaagcccccgccagtgtcagagatgatccgagagatgtgtccagccagtgggcctcctctgtgaaccagatgcatccggggacaggccaggcccgccgagagcagcagatcctgcccagggtcgctgcactgtccaggaggcagggagaggactttctgctacacaagagtattgacgtaacaggtgacccaaactctccgagacccaagcagaccttggagaaggatctgaaggaaaacagggaagagaacccaggactgtcatccccagagcctcagcttagagacgtat

SEQ ID NO: 26 - DNA, 793 bp, synthetic construct
  source 1..793: mol_type = other DNA; note = ZSCAN5B, gene synthesis fragment 2, coding aa243-495
tcacgtctcagcttccaaagagtcccaatctggtgagagcaaaggaggggaaggaaccccagaaaagagcctctgtggaaaatgtggatgctgacacaccttctgcctgcgttgtggagagagaagctttgactcacagcgggaacagaggagatgctctgaatctgagcagtcccaaaagaagcaaaccagatgcctcctccatttcccaagaagagcctcaaggagaagccacacctgtgggcaacagagaatccccaggacaagctgagatcaatccagttcattccccaggccctgcgggcccggtcagtcacccagatggccaagaagccaaggccctgccgccctttgcatgtgacgtgtgcaataaatcatttaagtatttttcccagctaagcatccacaggaggtcacacacaggagacagaccctttcaatgtgatctctgtcggaagcgcttcttgcagccctcagacctccgagttcaccagcgagtccacactggcgagaggccctacatgtgtgacgtctgccaaaagcggttcgcccacgagtccaccttacagggccacaagaggatccacaccggggagaggccgtttaaatgtaaatactgcagcaaagttttcagccacaaggggaacctgaacgttcaccagcgcacccactccggagagaagccctacaaatgtcccacctgtcaaaaggccttccgtcagctggggacattcaagcgtcacctgaaaacacaccgggaaaccacctcccagtgataatcgacgagacgcat

SEQ ID NO: 27 - DNA, 32 bp, synthetic construct
  source 1..32: mol_type = other DNA; note = sense ZSCAN5B-F3
atacgtctcacatggctgcaaattggacactc

SEQ ID NO: 28 - DNA, 43 bp, synthetic construct
  source 1..43: mol_type = other DNA; note = asense ZSCAN5B-F3
atacgtctcatcgagctgggaggtggtttcccggtgtgttttc

SEQ ID NO: 29 - DNA, 788 bp, synthetic construct
  source 1..788: mol_type = other DNA; note = ZSCAN5B -PCR-fragment-3 without Stop-Codon
tcacgtctcagcttccaaagagtcccaatctggtgagagcaaaggaggggaaggaaccccagaaaagagcctctgtggaaaatgtggatgctgacacaccttctgcctgcgttgtggagagagaagctttgactcacagcgggaacagaggagatgctctgaatctgagcagtcccaaaagaagcaaaccagatgcctcctccatttcccaagaagagcctcaaggagaagccacacctgtgggcaacagagaatccccaggacaagctgagatcaatccagttcattccccaggccctgcgggcccggtcagtcacccagatggccaagaagccaaggccctgccgccctttgcatgtgacgtgtgcaataaatcatttaagtatttttcccagctaagcatccacaggaggtcacacacaggagacagaccctttcaatgtgatctctgtcggaagcgcttcttgcagccctcagacctccgagttcaccagcgagtccacactggcgagaggccctacatgtgtgacgtctgccaaaagcggttcgcccacgagtccaccttacagggccacaagaggatccacaccggggagaggccgtttaaatgtaaatactgcagcaaagttttcagccacaaggggaacctgaacgttcaccagcgcacccactccggagagaagccctacaaatgtcccacctgtcaaaaggccttccgtcagctggggacattcaagcgtcacctgaaaacacaccgggaaaccacctcccagctcgatgagacgtat

SEQ ID NO: 30 - DNA, 7104 bp, synthetic construct
  source 1..7104: mol_type = other DNA; note = pTriEx-1-ZSCAN5B [human]
ggagtcgctgcgacgctgccttcgccccgtgccccgctccgccgccgcctcgcgccgcccgccccggctctgactgaccgcgttactcccacaggtgagcgggcgggacggcccttctccttcgggctgtaattagcgcttggtttaatgacggcttgtttcttttctgtggctgcgtgaaagccttgaggggctccgggagggccctttgtgcggggggagcggctcggggctgtccgcggggggacggctgccttcgggggggacggggcagggcggggttcggcttctggcgtgtgaccggcggctctagagcctctgctaaccatgttcatgccttcttctttttcctacagctcctgggcaacgtgctggttattgtgctgtctcatcattttggcaaagaattggatcggaccgaaattaatacgactcactataggggaattgtgagcggataacaattccccggagttaatccgggacctttaattcaacccaacacaatatattatagttaaataagaattattatcaaatcatttgtatattaattaaaatactatactgtaaattacattttatttacaatcaaaggagatataccatggctgcaaattggacactctcatggggtcagggaggaccctgcaacagccctgggtcagacactccacggtctgtggcgtccccagaaactcaacttggaaatcacgacaggaaccctgagacttggcacatgaatttcaggatgttcagctgcccagaggagtcggaccccatccaggctctgaggaaactcactgagctgtgccatctgtggctgaggcccgacctccacaccaaagagcagatcctggacatgctggtgatggagcagttcatgatctccatgccccaggagctccaggtcttagtcaaggtgaacggtgtgcagagctgcaaagacctggaggacctgctacgaaataacagaagacccaagaaatggtctatagtcaacttgctcggcaaagaatatcttatgctgaactcagatgtcgagatggctgaagcccccgccagtgtcagagatgatccgagagatgtgtccagccagtgggcctcctctgtgaaccagatgcatccggggacaggccaggcccgccgagagcagcagatcctgcccagggtcgctgcactgtccaggaggcagggagaggactttctgctacacaagagtattgacgtaacaggtgacccaaactctccgagacccaagcagaccttggagaaggatctgaaggaaaacagggaagagaacccaggactgtcatccccagagcctcagcttccaaagagtcccaatctggtgagagcaaaggaggggaaggaaccccagaaaagagcctctgtggaaaatgtggatgctgacacaccttctgcctgcgttgtggagagagaagctttgactcacagcgggaacagaggagatgctctgaatctgagcagtcccaaaagaagcaaaccagatgcctcctccatttcccaagaagagcctcaaggagaagccacacctgtgggcaacagagaatccccaggacaagctgagatcaatccagttcattccccaggccctgcgggcccggtcagtcacccagatggccaagaagccaaggccctgccgccctttgcatgtgacgtgtgcaataaatcatttaagtatttttcccagctaagcatccacaggaggtcacacacaggagacagaccctttcaatgtgatctctgtcggaagcgcttcttgcagccctcagacctccgagttcaccagcgagtccacactggcgagaggccctacatgtgtgacgtctgccaaaagcggttcgcccacgagtccaccttacagggccacaagaggatccacaccggggagaggccgtttaaatgtaaatactgcagcaaagttttcagccacaaggggaacctgaacgttcaccagcgcacccactccggagagaagccctacaaatgtcccacctgtcaaaaggccttccgtcagctggggacattcaagcgtcacctgaaaacacaccgggaaaccacctcccagtgataatcgagcaccaccatcaccatcaccatcactaagtgattaacctcaggtgcaggctgcctatcagaaggtggtggctggtgtggccaatgccctggctcacaaataccactgagatcgatctttttccctctgccaaaaattatggggacatcatgaagccccttgagcatctgacttctggctaataaaggaaatttattttcattgcaatagtgtgttggaattttttgtgtctctcactcggaaggacatatgggagggcaaatcatttaaaacatcagaatgagtatttggtttagagtttggcaacatatgcccatatgtaactagcataaccccttggggcctctaaacgggtcttgaggggttttttgctgaaagcatgcggaggaaattctccttgaagtttccctggtgttcaaagtaaaggagtttgcaccagacgcacctctgttcactggtccggcgtattaaaacacgatacattgttattagtacatttattaagcgctagattctgtgcgttgttgatttacagacaattgttgtacgtattttaataattcattaaatttataatctttagggtggtatgttagagcgaaaatcaaatgattttcagcgtctttatatctgaatttaaatattaaatcctcaatagatttgtaaaataggtttcgattagtttcaaacaagggttgtttttccgaaccgatggctggactatctaatggattttcgctcaacgccacaaaacttgccaaatcttgtagcagcaatctagctttgtcgatattcgtttgtgttttgttttgtaataaaggttcgacgtcgttcaaaatattatgcgcttttgtatttctttcatcactgtcgttagtgtacaattgactcgacgtaaacacgttaaatagagcttggacatatttaacatcgggcgtgttagctttattaggccgattatcgtcgtcgtcccaaccctcgtcgttagaagttgcttccgaagacgattttgccatagccacacgacgcctattaattgtgtcggctaacacgtccgcgatcaaatttgtagttgagctttttggaattatttctgattgcgggcgtttttgggcgggtttcaatctaactgtgcccgattttaattcagacaacacgttagaaagcgatggtgcaggcggtggtaacatttcagacggcaaatctactaatggcggcggtggtggagctgatgataaatctaccatcggtggaggcgcaggcggggctggcggcggaggcggaggcggaggtggtggcggtgatgcagacggcggtttaggctcaaatgtctctttaggcaacacagtcggcacctcaactattgtactggtttcgggcgccgtttttggtttgaccggtctgagacgagtgcgatttttttcgtttctaatagcttccaacaattgttgtctgtcgtctaaaggtgcagcgggttgaggttccgtcggcattggtggagcgggcggcaattcagacatcgatggtggtggtggtggtggaggcgctggaatgttaggcacgggagaaggtggtggcggcggtgccgccggtataatttgttctggtttagtttgttcgcgcacgattgtgggcaccggcgcaggcgccgctggctgcacaacggaaggtcgtctgcttcgaggcagcgcttggggtggtggcaattcaatattataattggaatacaaatcgtaaaaatctgctataagcattgtaatttcgctatcgtttaccgtgccgatatttaacaaccgctcaatgtaagcaattgtattgtaaagagattgtctcaagctcggaacgctgcgctcggtcgttcggctgcggcgagcggtatcagctcactcaaaggcggtaatacggttatccacagaatcaggggataacgcaggaaagaacatgtgagcaaaaggccagcaaaaggccaggaaccgtaaaaaggccgcgttgctggcgtttttccataggctccgcccccctgacgagcatcacaaaaatcgacgctcaagtcagaggtggcgaaacccgacaggactataaagataccaggcgtttccccctggaagctccctcgtgcgctctcctgttccgaccctgccgcttaccggatacctgtccgcctttctcccttcgggaagcgtggcgctttctcaatgctcacgctgtaggtatctcagttcggtgtaggtcgttcgctccaagctgggctgtgtgcacgaaccccccgttcagcccgaccgctgcgccttatccggtaactatcgtcttgagtccaacccggtaagacacgacttatcgccactggcagcagccactggtaacaggattagcagagcgaggtatgtaggcggtgctacagagttcttgaagtggtggcctaactacggctacactagaaggacagtatttggtatctgcgctctgctgaagccagttaccttcggaaaaagagttggtagctcttgatccggcaaacaaaccaccgctggtagcggtggtttttttgtttgcaagcagcagattacgcgcagaaaaaaaggatctcaagaagatcctttgttaccaatgcttaatcagtgaggcacctatctcagcgatctgtctatttcgttcatccatagttgcctgactccccgtcgtgtagataactacgatacgggagggcttaccatctggccccagtgctgcaatgataccgcgagacccacgctcaccggctccagatttatcagcaataaaccagccagccggaagggccgagcgcagaagtggtcctgcaactttatccgcctccatccagtctattaattgttgccgggaagctagagtaagtagttcgccagttaatagtttgcgcaacgttgttgccattgctacaggcatcgtggtgtcacgctcgtcgtttggtatggcttcattcagctccggttcccaacgatcaaggcgagttacatgatcccccatgttgtgcaaaaaagcggttagctccttcggtcctccgatcgttgtcagaagtaagttggccgcagtgttatcactcatggttatggcagcactgcataattctcttactgtcatgccatccgtaagatgcttttctgtgactggtgagtactcaaccaagtcattctgagaatagtgtatgcggcgaccgagttgctcttgcccggcgtcaatacgggataataccgcgccacatagcagaactttaaaagtgctcatcattggaaaacgttcttcggggcgaaaactctcaaggatcttaccgctgttgagatccagttcgatgtaacccactcgtgcacccaactgatcttcagcatcttttactttcaccagcgtttctgggtgagcaaaaacaggaaggcaaaatgccgcaaaaaagggaataagggcgacacggaaatgttgaatactcatactcttcctttttcaatattattgaagcatttatcagggttattgtctcatgtccgcgcgtttcctgcatcttttaatcaaatcccaagatgtgtataaaccaccaaactgccaaaaaatgaaaactgtcgacaagctctgtccgtttgctggcaactgcaagggtctcaatcctatttgtaattattgaataataaaacaattataaatgtcaaatttgttttttattaacgatacaaaccaaacgcaacaagaacatttgtagtattatctataattgaaaacgcgtagttataatcgctgaggtaatatttaaaatcattttcaaatgattcacagttaatttgcgacaatataattttattttcacataaactagacgccttgtcgtcttcttcttcgtattccttctctttttcatttttctcttcataaaaattaacatagttattatcgtatccatatatgtatctatcgtatagagtaaattttttgttgtcataaatatatatgtcttttttaatggggtgtatagtaccgctgcgcatagtttttctgtaatttacaacagtgctattttctggtagttcttcggagtgtgttgctttaattattaaatttatataatcaatgaatttgggatcgtcggttttgtacaatatgttgccggcatagtacgcagcttcttctagttcaattacaccattttttagcagcaccggattaacataactttccaaaatgttgtacgaaccgttaaacaaaaacagttcacctcccttttctatactattgtctgcgagcagttgtttgttgttaaaaataacagccattgtaatgagacgcacaaactaatatcacaaactggaaatgtctatcaatatatagttgctctagttattaatagtaatcaattacggggtcattagttcatagcccatatatggagttccgcgttacataacttacggtaaatggcccgcctggctgaccgcccaacgacccccgcccattgacgtcaataatgacgtatgttcccatagtaacgccaatagggactttccattgacgtcaatgggtggactatttacggtaaactgcccacttggcagtacatcaagtgtatcatatgccaagtacgccccctattgacgtcaatgacggtaaatggcccgcctggcattatgcccagtacatgaccttatgggactttcctacttggcagtacatctacgtattagtcatcgctattaccatgcatggtcgaggtgagccccacgttctgcttcactctccccatctcccccccctccccacccccaattttgtatttatttattttttaattattttgtgcagcgatgggggcggggggggggggggggcgcgcgccaggcggggcggggcggggcgaggggcggggcggggcgaggcggagaggtgcggcggcagccaatcagagcggcgcgctccgaaagtttccttttatggcgaggcggcggcggcggcggccctataaaaagcgaagcgcgcggcgggcg

SEQ ID NO: 31 - protein, 495 aa, Homo sapiens; identical to SEQ ID NO: 6
  source 1..495: note = ZSCAN5B[human]

SEQ ID NO: 32 - DNA, 7099 bp, synthetic construct
  source 1..7099: mol_type = other DNA; note = pTriEx-1-ZSCAN5B[human]-His
ggagtcgctgcgacgctgccttcgccccgtgccccgctccgccgccgcctcgcgccgcccgccccggctctgactgaccgcgttactcccacaggtgagcgggcgggacggcccttctccttcgggctgtaattagcgcttggtttaatgacggcttgtttcttttctgtggctgcgtgaaagccttgaggggctccgggagggccctttgtgcggggggagcggctcggggctgtccgcggggggacggctgccttcgggggggacggggcagggcggggttcggcttctggcgtgtgaccggcggctctagagcctctgctaaccatgttcatgccttcttctttttcctacagctcctgggcaacgtgctggttattgtgctgtctcatcattttggcaaagaattggatcggaccgaaattaatacgactcactataggggaattgtgagcggataacaattccccggagttaatccgggacctttaattcaacccaacacaatatattatagttaaataagaattattatcaaatcatttgtatattaattaaaatactatactgtaaattacattttatttacaatcaaaggagatataccatggctgcaaattggacactctcatggggtcagggaggaccctgcaacagccctgggtcagacactccacggtctgtggcgtccccagaaactcaacttggaaatcacgacaggaaccctgagacttggcacatgaatttcaggatgttcagctgcccagaggagtcggaccccatccaggctctgaggaaactcactgagctgtgccatctgtggctgaggcccgacctccacaccaaagagcagatcctggacatgctggtgatggagcagttcatgatctccatgccccaggagctccaggtcttagtcaaggtgaacggtgtgcagagctgcaaagacctggaggacctgctacgaaataacagaagacccaagaaatggtctatagtcaacttgctcggcaaagaatatcttatgctgaactcagatgtcgagatggctgaagcccccgccagtgtcagagatgatccgagagatgtgtccagccagtgggcctcctctgtgaaccagatgcatccggggacaggccaggcccgccgagagcagcagatcctgcccagggtcgctgcactgtccaggaggcagggagaggactttctgctacacaagagtattgacgtaacaggtgacccaaactctccgagacccaagcagaccttggagaaggatctgaaggaaaacagggaagagaacccaggactgtcatccccagagcctcagcttccaaagagtcccaatctggtgagagcaaaggaggggaaggaaccccagaaaagagcctctgtggaaaatgtggatgctgacacaccttctgcctgcgttgtggagagagaagctttgactcacagcgggaacagaggagatgctctgaatctgagcagtcccaaaagaagcaaaccagatgcctcctccatttcccaagaagagcctcaaggagaagccacacctgtgggcaacagagaatccccaggacaagctgagatcaatccagttcattccccaggccctgcgggcccggtcagtcacccagatggccaagaagccaaggccctgccgccctttgcatgtgacgtgtgcaataaatcatttaagtatttttcccagctaagcatccacaggaggtcacacacaggagacagaccctttcaatgtgatctctgtcggaagcgcttcttgcagccctcagacctccgagttcaccagcgagtccacactggcgagaggccctacatgtgtgacgtctgccaaaagcggttcgcccacgagtccaccttacagggccacaagaggatccacaccggggagaggccgtttaaatgtaaatactgcagcaaagttttcagccacaaggggaacctgaacgttcaccagcgcacccactccggagagaagccctacaaatgtcccacctgtcaaaaggccttccgtcagctggggacattcaagcgtcacctgaaaacacaccgggaaaccacctcccagctcgagcaccaccatcaccatcaccatcactaagtgattaacctcaggtgcaggctgcctatcagaaggtggtggctggtgtggccaatgccctggctcacaaataccactgagatcgatctttttccctctgccaaaaattatggggacatcatgaagccccttgagcatctgacttctggctaataaaggaaatttattttcattgcaatagtgtgttggaattttttgtgtctctcactcggaaggacatatgggagggcaaatcatttaaaacatcagaatgagtatttggtttagagtttggcaacatatgcccatatgtaactagcataaccccttggggcctctaaacgggtcttgaggggttttttgctgaaagcatgcggaggaaattctccttgaagtttccctggtgttcaaagtaaaggagtttgcaccagacgcacctctgttcactggtccggcgtattaaaacacgatacattgttattagtacatttattaagcgctagattctgtgcgttgttgatttacagacaattgttgtacgtattttaataattcattaaatttataatctttagggtggtatgttagagcgaaaatcaaatgattttcagcgtctttatatctgaatttaaatattaaatcctcaatagatttgtaaaataggtttcgattagtttcaaacaagggttgtttttccgaaccgatggctggactatctaatggattttcgctcaacgccacaaaacttgccaaatcttgtagcagcaatctagctttgtcgatattcgtttgtgttttgttttgtaataaaggttcgacgtcgttcaaaatattatgcgcttttgtatttctttcatcactgtcgttagtgtacaattgactcgacgtaaacacgttaaatagagcttggacatatttaacatcgggcgtgttagctttattaggccgattatcgtcgtcgtcccaaccctcgtcgttagaagttgcttccgaagacgattttgccatagccacacgacgcctattaattgtgtcggctaacacgtccgcgatcaaatttgtagttgagctttttggaattatttctgattgcgggcgtttttgggcgggtttcaatctaactgtgcccgattttaattcagacaacacgttagaaagcgatggtgcaggcggtggtaacatttcagacggcaaatctactaatggcggcggtggtggagctgatgataaatctaccatcggtggaggcgcaggcggggctggcggcggaggcggaggcggaggtggtggcggtgatgcagacggcggtttaggctcaaatgtctctttaggcaacacagtcggcacctcaactattgtactggtttcgggcgccgtttttggtttgaccggtctgagacgagtgcgatttttttcgtttctaatagcttccaacaattgttgtctgtcgtctaaaggtgcagcgggttgaggttccgtcggcattggtggagcgggcggcaattcagacatcgatggtggtggtggtggtggaggcgctggaatgttaggcacgggagaaggtggtggcggcggtgccgccggtataatttgttctggtttagtttgttcgcgcacgattgtgggcaccggcgcaggcgccgctggctgcacaacggaaggtcgtctgcttcgaggcagcgcttggggtggtggcaattcaatattataattggaatacaaatcgtaaaaatctgctataagcattgtaatttcgctatcgtttaccgtgccgatatttaacaaccgctcaatgtaagcaattgtattgtaaagagattgtctcaagctcggaacgctgcgctcggtcgttcggctgcggcgagcggtatcagctcactcaaaggcggtaatacggttatccacagaatcaggggataacgcaggaaagaacatgtgagcaaaaggccagcaaaaggccaggaaccgtaaaaaggccgcgttgctggcgtttttccataggctccgcccccctgacgagcatcacaaaaatcgacgctcaagtcagaggtggcgaaacccgacaggactataaagataccaggcgtttccccctggaagctccctcgtgcgctctcctgttccgaccctgccgcttaccggatacctgtccgcctttctcccttcgggaagcgtggcgctttctcaatgctcacgctgtaggtatctcagttcggtgtaggtcgttcgctccaagctgggctgtgtgcacgaaccccccgttcagcccgaccgctgcgccttatccggtaactatcgtcttgagtccaacccggtaagacacgacttatcgccactggcagcagccactggtaacaggattagcagagcgaggtatgtaggcggtgctacagagttcttgaagtggtggcctaactacggctacactagaaggacagtatttggtatctgcgctctgctgaagccagttaccttcggaaaaagagttggtagctcttgatccggcaaacaaaccaccgctggtagcggtggtttttttgtttgcaagcagcagattacgcgcagaaaaaaaggatctcaagaagatcctttgttaccaatgcttaatcagtgaggcacctatctcagcgatctgtctatttcgttcatccatagttgcctgactccccgtcgtgtagataactacgatacgggagggcttaccatctggccccagtgctgcaatgataccgcgagacccacgctcaccggctccagatttatcagcaataaaccagccagccggaagggccgagcgcagaagtggtcctgcaactttatccgcctccatccagtctattaattgttgccgggaagctagagtaagtagttcgccagttaatagtttgcgcaacgttgttgccattgctacaggcatcgtggtgtcacgctcgtcgtttggtatggcttcattcagctccggttcccaacgatcaaggcgagttacatgatcccccatgttgtgcaaaaaagcggttagctccttcggtcctccgatcgttgtcagaagtaagttggccgcagtgttatcactcatggttatggcagcactgcataattctcttactgtcatgccatccgtaagatgcttttctgtgactggtgagtactcaaccaagtcattctgagaatagtgtatgcggcgaccgagttgctcttgcccggcgtcaatacgggataataccgcgccacatagcagaactttaaaagtgctcatcattggaaaacgttcttcggggcgaaaactctcaaggatcttaccgctgttgagatccagttcgatgtaacccactcgtgcacccaactgatcttcagcatcttttactttcaccagcgtttctgggtgagcaaaaacaggaaggcaaaatgccgcaaaaaagggaataagggcgacacggaaatgttgaatactcatactcttcctttttcaatattattgaagcatttatcagggttattgtctcatgtccgcgcgtttcctgcatcttttaatcaaatcccaagatgtgtataaaccaccaaactgccaaaaaatgaaaactgtcgacaagctctgtccgtttgctggcaactgcaagggtctcaatcctatttgtaattattgaataataaaacaattataaatgtcaaatttgttttttattaacgatacaaaccaaacgcaacaagaacatttgtagtattatctataattgaaaacgcgtagttataatcgctgaggtaatatttaaaatcattttcaaatgattcacagttaatttgcgacaatataattttattttcacataaactagacgccttgtcgtcttcttcttcgtattccttctctttttcatttttctcttcataaaaattaacatagttattatcgtatccatatatgtatctatcgtatagagtaaattttttgttgtcataaatatatatgtcttttttaatggggtgtatagtaccgctgcgcatagtttttctgtaatttacaacagtgctattttctggtagttcttcggagtgtgttgctttaattattaaatttatataatcaatgaatttgggatcgtcggttttgtacaatatgttgccggcatagtacgcagcttcttctagttcaattacaccattttttagcagcaccggattaacataactttccaaaatgttgtacgaaccgttaaacaaaaacagttcacctcccttttctatactattgtctgcgagcagttgtttgttgttaaaaataacagccattgtaatgagacgcacaaactaatatcacaaactggaaatgtctatcaatatatagttgctctagttattaatagtaatcaattacggggtcattagttcatagcccatatatggagttccgcgttacataacttacggtaaatggcccgcctggctgaccgcccaacgacccccgcccattgacgtcaataatgacgtatgttcccatagtaacgccaatagggactttccattgacgtcaatgggtggactatttacggtaaactgcccacttggcagtacatcaagtgtatcatatgccaagtacgccccctattgacgtcaatgacggtaaatggcccgcctggcattatgcccagtacatgaccttatgggactttcctacttggcagtacatctacgtattagtcatcgctattaccatgcatggtcgaggtgagccccacgttctgcttcactctccccatctcccccccctccccacccccaattttgtatttatttattttttaattattttgtgcagcgatgggggcggggggggggggggggcgcgcgccaggcggggcggggcggggcgaggggcggggcggggcgaggcggagaggtgcggcggcagccaatcagagcggcgcgctccgaaagtttccttttatggcgaggcggcggcggcggcggccctataaaaagcgaagcgcgcggcgggcg

SEQ ID NO: 33 - protein, 505 aa, synthetic construct
  source 1..505: note = VGLUT2[human]-H8
MAANWTLSWGQGGPCNSPGSDTPRSVASPETQLGNHDRNPETWHMNFRMFSCPEESDPIQALRKLTELCHLWLRPDLHTKEQILDMLVMEQFMISMPQELQVLVKVNGVQSCKDLEDLLRNNRRPKKWSIVNLLGKEYLMLNSDVEMAEAPASVRDDPRDVSSQWASSVNQMHPGTGQARREQQILPRVAALSRRQGEDFLLHKSIDVTGDPNSPRPKQTLEKDLKENREENPGLSSPEPQLPKSPNLVRAKEGKEPQKRASVENVDADTPSACVVEREALTHSGNRGDALNLSSPKRSKPDASSISQEEPQGEATPVGNRESPGQAEINPVHSPGPAGPVSHPDGQEAKALPPFACDVCNKSFKYFSQLSIHRRSHTGDRPFQCDLCRKRFLQPSDLRVHQRVHTGERPYMCDVCQKRFAHESTLQGHKRIHTGERPFKCKYCSKVFSHKGNLNVHQRTHSGEKPYKCPTCQKAFRQLGTFKRHLKTHRETTSQLEHHHHHHHH

SEQ ID NO: 34 - protein, 203 aa, synthetic construct
  source 1..203: note = GamS-ZSCAN5A-6His
MGNAYYIQDRLEAQSWARHYQQLAREEKEAELADDMEKGLPQHLFESLCIDHLQRHGASKKSITRAFDDDVEFQERMAEHIRYMVETIAHHQVDIDSEVGGSGTPSACVVEREASTHSGSRGDALNLRGLKRSKPDATSISQEEPQGEATPVGNRESPGQAEINPVHSPGPAGPVSHPSGQEVKELLPFACEVGGSGHHHHHH

SEQ ID NO: 35 - protein, 201 aa, synthetic construct
  source 1..201: note = GamS-ZSCAN5B-6His
MGNAYYIQDRLEAQSWARHYQQLAREEKEAELADDMEKGLPQHLFESLCIDHLQRHGASKKSITRAFDDDVEFQERMAEHIRYMVETIAHHQVDIDSEVGGSGSACVVEREALTHSGNRGDALNLSSPKRSKPDASSISQEEPQGEATPVGNRESPGQAEINPVHSPGPAGPVSHPDGQEAKALPPFACDVGGSGHHHHHH

SEQ ID NO: 36 - protein, 203 aa, synthetic construct
  source 1..203: note = GamS-ZSCAN5C-6His
MGNAYYIQDRLEAQSWARHYQQLAREEKEAELADDMEKGLPQHLFESLCIDHLQRHGASKKSITRAFDDDVEFQERMAEHIRYMVETIAHHQVDIDSEVGGSGTPSACVVEREASTHSGNRGDALNLSSPKRSKPDASSISQEEPQGEATPVGNRESPGQAGMNSIHSPGPASPVSHPDGQEAKALPPFACDVGGSGHHHHHH

SEQ ID NO: 37 - DNA, 1730 bp, synthetic construct
  source 1..1730: mol_type = other DNA; note = GamS-ZSCAN5A-6His gene fragment with adapters
gaggtgacgggcctcaaagccgcgtgggagtgagctaacaccgtgcgtgttgacaattttacctctggcggtgataatggttgcagctactaataattttgtttaactttaagaaggagatataccatgggaaacgcttattacattcaggatcgtcttgaggctcagagctgggcgcgtcactaccagcagctcgcccgtgaagagaaagaggcagaactggcagacgacatggaaaaaggcctgccccagcacctgtttgaatcgctatgcatcgatcatttgcaacgccacggggccagcaaaaaatccattacccgtgcgtttgatgacgatgttgagtttcaggagcgcatggcagaacacatccggtacatggttgaaaccattgctcaccaccaggttgatattgattcagaggtaggtggtagcggtactccgagcgcatgtgtggtggaacgagaagcatcgacacattcagggagcagaggggacgccctgaatttacgtggcctcaaacgttccaaacccgatgctacttctattagccaagaggaaccgcaaggagaggcaacaccggtaggcaaccgtgaatctcctggccaggcagagatcaaccctgttcactcccctggtcccgctggtccggtttctcatccgagcgggcaggaggtcaaagaacttcttccatttgcgtgtgaagtaggtggtagcggtcatcatcaccatcatcattaaaatgcaaagcccgccgaaaggcgggcttttctgtacttcgcaacgatttcggagtccggagactcgctgttttcgaaatttgcgctcaagggcgggtattgaacccaatccgccctcactacaaccggaggtgacgggcctcaaagccgcgtgggagtgagctaacaccgtgcgtgttgacaattttacctctggcggtgataatggttgcagctactaataattttgtttaactttaagaaggagatataccatgggaaacgcttattacattcaggatcgtcttgaggctcagagctgggcgcgtcactaccagcagctcgcccgtgaagagaaagaggcagaactggcagacgacatggaaaaaggcctgccccagcacctgtttgaatcgctatgcatcgatcatttgcaacgccacggggccagcaaaaaatccattacccgtgcgtttgatgacgatgttgagtttcaggagcgcatggcagaacacatccggtacatggttgaaaccattgctcaccaccaggttgatattgattcagaggtaggtggtagcggtactccgagcgcatgtgtggtggaacgagaagcatcgacacattcagggagcagaggggacgccctgaatttacgtggcctcaaacgttccaaacccgatgctacttctattagccaagaggaaccgcaaggagaggcaacaccggtaggcaaccgtgaatctcctggccaggcagagatcaaccctgttcactcccctggtcccgctggtccggtttctcatccgagcgggcaggaggtcaaagaacttcttccatttgcgtgtgaagtaggtggtagcggtcatcatcaccatcatcattaaaatgcaaagcccgccgaaaggcgggcttttctgtacttcgcaacgatttcggagtccggagactcgctgttttcgaaatttgcgctcaagggcgggtattgaaccctactctggcgtcgatgaggga

SEQ ID NO: 38 - DNA, 1718 bp, synthetic construct
  source 1..1718: mol_type = other DNA; note = GamS-ZSCAN5B-6His gene fragment with adapters
gaggtgacgggcctcaaagccgcgtgggagtgagctaacaccgtgcgtgttgacaattttacctctggcggtgataatggttgcagctactaataattttgtttaactttaagaaggagatataccatgggaaacgcttattacattcaggatcgtcttgaggctcagagctgggcgcgtcactaccagcagctcgcccgtgaagagaaagaggcagaactggcagacgacatggaaaaaggcctgccccagcacctgtttgaatcgctatgcatcgatcatttgcaacgccacggggccagcaaaaaatccattacccgtgcgtttgatgacgatgttgagtttcaggagcgcatggcagaacacatccggtacatggttgaaaccattgctcaccaccaggttgatattgattcagaggtaggtggtagcggttctgcttgtgttgtggaacgggaagcgctgactcatagtggcaatcgcggtgacgcactcaatcttagcagccccaaacgcagcaagccggacgcgtctagcattagccaggaagaaccgcagggagaagcaactcctgttggcaaccgagaatcccctgggcaagccgaaatcaatcctgtacactctccgggacctgcaggccccgtttcacatccggatggacaagaggcgaaagcactcccgccgttcgcatgcgatgtgggtggtagcggtcatcatcaccatcatcattaaaatgcaaagcccgccgaaaggcgggcttttctgtacttcgcaacgatttcggagtccggagactcgctgttttcgaaatttgcgctcaagggcgggtattgaacccaatccgccctcactacaaccggaggtgacgggcctcaaagccgcgtgggagtgagctaacaccgtgcgtgttgacaattttacctctggcggtgataatggttgcagctactaataattttgtttaactttaagaaggagatataccatgggaaacgcttattacattcaggatcgtcttgaggctcagagctgggcgcgtcactaccagcagctcgcccgtgaagagaaagaggcagaactggcagacgacatggaaaaaggcctgccccagcacctgtttgaatcgctatgcatcgatcatttgcaacgccacggggccagcaaaaaatccattacccgtgcgtttgatgacgatgttgagtttcaggagcgcatggcagaacacatccggtacatggttgaaaccattgctcaccaccaggttgatattgattcagaggtaggtggtagcggttctgcttgtgttgtggaacgggaagcgctgactcatagtggcaatcgcggtgacgcactcaatcttagcagccccaaacgcagcaagccggacgcgtctagcattagccaggaagaaccgcagggagaagcaactcctgttggcaaccgagaatcccctgggcaagccgaaatcaatcctgtacactctccgggacctgcaggccccgtttcacatccggatggacaagaggcgaaagcactcccgccgttcgcatgcgatgtgggtggtagcggtcatcatcaccatcatcattaaaatgcaaagcccgccgaaaggcgggcttttctgtacttcgcaacgatttcggagtccggagactcgctgttttcgaaatttgcgctcaagggcgggtattgaaccctactctggcgtcgatgaggga

SEQ ID NO: 39 - DNA, 1730 bp, synthetic construct
  source 1..1730: mol_type = other DNA; note = GamS-ZSCAN5C-6His gene fragment with adapters
gaggtgacgggcctcaaagccgcgtgggagtgagctaacaccgtgcgtgttgacaattttacctctggcggtgataatggttgcagctactaataattttgtttaactttaagaaggagatataccatgggaaacgcttattacattcaggatcgtcttgaggctcagagctgggcgcgtcactaccagcagctcgcccgtgaagagaaagaggcagaactggcagacgacatggaaaaaggcctgccccagcacctgtttgaatcgctatgcatcgatcatttgcaacgccacggggccagcaaaaaatccattacccgtgcgtttgatgacgatgttgagtttcaggagcgcatggcagaacacatccggtacatggttgaaaccattgctcaccaccaggttgatattgattcagaggtaggtggtagcggtaccccaagcgcttgtgtagtcgaaagagaagcaagtacgcacagcggcaatcggggggacgccttgaacttgtcttctcctaaaagatcgaagcccgatgcgtcatcaattagccaggaagaaccacagggtgaagcgacaccggtaggcaatagagagtctcctggacaagccggaatgaactcgatccattccccgggcccagcatcaccggtgagccacccggatggccaggaggcgaaggccctgccaccatttgcctgcgatgttggtggtagcggtcatcatcaccatcatcattaaaatgcaaagcccgccgaaaggcgggcttttctgtacttcgcaacgatttcggagtccggagactcgctgttttcgaaatttgcgctcaagggcgggtattgaacccaatccgccctcactacaaccggaggtgacgggcctcaaagccgcgtgggagtgagctaacaccgtgcgtgttgacaattttacctctggcggtgataatggttgcagctactaataattttgtttaactttaagaaggagatataccatgggaaacgcttattacattcaggatcgtcttgaggctcagagctgggcgcgtcactaccagcagctcgcccgtgaagagaaagaggcagaactggcagacgacatggaaaaaggcctgccccagcacctgtttgaatcgctatgcatcgatcatttgcaacgccacggggccagcaaaaaatccattacccgtgcgtttgatgacgatgttgagtttcaggagcgcatggcagaacacatccggtacatggttgaaaccattgctcaccaccaggttgatattgattcagaggtaggtggtagcggtaccccaagcgcttgtgtagtcgaaagagaagcaagtacgcacagcggcaatcggggggacgccttgaacttgtcttctcctaaaagatcgaagcccgatgcgtcatcaattagccaggaagaaccacagggtgaagcgacaccggtaggcaatagagagtctcctggacaagccggaatgaactcgatccattccccgggcccagcatcaccggtgagccacccggatggccaggaggcgaaggccctgccaccatttgcctgcgatgttggtggtagcggtcatcatcaccatcatcattaaaatgcaaagcccgccgaaaggcgggcttttctgtacttcgcaacgatttcggagtccggagactcgctgttttcgaaatttgcgctcaagggcgggtattgaaccctactctggcgtcgatgaggga

SEQ ID NO: 40 - protein, 90 aa, synthetic construct
  source 1..90: note = epitope from ZSCAN5A
TPSACVVEREASTHSGNRGDALNLSSPKRSKPDASSISQEEPQGEATPVGNRESPGQAGMNSIHSPGPASPVSHPDGQEAKALPPFACDV

SEQ ID NO: 41 - protein, 89 aa, synthetic construct
  source 1..89: note = epitope from ZSCAN5B
SACVVEREALTHSGNRGDALNLSSPKRSKPDASSISQEEPQGEATPVGNRESPGQAEINPVHSPGPAGPVSHPDGQEAKALPPFACDVC

SEQ ID NO: 42 - protein, 90 aa, synthetic construct
  source 1..90: note = epitope from ZSCAN5C
TPSACVVEREASTHSGSRGDALNLRGLKRSKPDATSISQEEPQGEATPVGNRESPGQAEINPVHSPGPAGPVSHPSGQEVKELLPFACEV

SEQ ID NO: 43 - protein, 353 aa, Homo sapiens
ASPTSPKVFPLSLCSTQPDGNVVIACLVQGFFPQEPLSVTWSESGQGVTARNFPPSQDASGDLYTTSSQLTLPATQCLAGKSVTCHVKHYTNPSQDVTVPCPVPSTPPTPSPSTPPTPSPSCCHPRLSLHRPALEDLLLGSEANLTCTLTGLRDASGVTFTWTPSSGKSAVQGPPERDLCGCYSVSSVLPGCAEPWNHGKTFTCTAAYPESKTPLTATLSKSGNTFRPEVHLLPPPSEELALNELVTLTCLARGFSPKDVLVRWLQGSQELPREKYLTWASRQEPSQGTTTFAVTSILRVAAEDWKKGDTFSCMVGHEALPLAFTQKTIDRLAGKPTHVNVSVVMAEVDGTCY

SEQ ID NO: 44 - protein, 340 aa, Homo sapiens
ASPTSPKVFPLSLDSTPQDGNVVVACLVQGFFPQEPLSVTWSESGQNVTARNFPPSQDASGDLYTTSSQLTLPATQCPDGKSVTCHVKHYTNSSQDVTVPCRVPPPPPCCHPRLSLHRPALEDLLLGSEANLTCTLTGLRDASGATFTWTPSSGKSAVQGPPERDLCGCYSVSSVLPGCAQPWNHGETFTCTAAHPELKTPLTANITKSGNTFRPEVHLLPPPSEELALNELVTLTCLARGFSPKDVLVRWLQGSQELPREKYLTWASRQEPSQGTTTYAVTSILRVAAEDWKKGETFSCMVGHEALPLAFTQKTIDRMAGKPTHINVSVVMAEADGTCY

SEQ ID NO: 45 - protein, 384 aa, Homo sapiens
APTKAPDVFPIISGCRHPKDNSPVVLACLITGYHPTSVTVTWYMGTQSQPQRTFPEIQRRDSYYMTSSQLSTPLQQWRQGEYKCVVQHTASKSKKEIFRWPESPKAQASSVPTAQPQAEGSLAKATTAPATTRNTGRGGEEKKKEKEKEEQEERETKTPECPSHTQPLGVYLLTPAVQDLWLRDKATFTCFVVGSDLKDAHLTWEVAGKVPTGGVEEGLLERHSNGSQSQHSRLTLPRSLWNAGTSVTCTLNHPSLPPQRLMALREPAAQAPVKLSLNLLASSDPPEAASWLLCEVSGFSPPNILLMWLEDQREVNTSGFAPARPPPQPRSTTFWAWSVLRVPAPPSPQPATYTCVVSHEDSRTLLNASRSLEVSYVTDHGPMK

SEQ ID NO: 46 - protein, 428 aa, Homo sapiens
ASTQSPSVFPLTRCCKNIPSNATSVTLGCLATGYFPEPVMVTWDTGSLNGTTMTLPATTLTLSGHYATISLLTVSGAWAKQMFTCRVAHTPSSTDWVDNKTFSVCSRDFTPPTVKILQSSCDGGGHFPPTIQLLCLVSGYTPGTINITWLEDGQVMDVDLSTASTTQEGELASTQSELTLSQKHWLSDRTYTCQVTYQGHTFEDSTKKCADSNPRGVSAYLSRPSPFDLFIRKSPTITCLVVDLAPSKGTVNLTWSRASGKPVNHSTRKEEKQRNGTLTVTSTLPVGTRDWIEGETYQCRVTHPHLPRALMRSTTKTSGPRAAPEVYAFATPEWPGSRDKRTLACLIQNFMPEDISVQWLHNEVQLPDARHSTTQPRKTKGSGFFVFSRLEVTRAEWEQKDEFICRAVHEAASPSQTVQRAVSVNPGK

SEQ ID NO: 47 - protein, 330 aa, Homo sapiens [sequence omitted]

SEQ ID NO: 48 - protein, 326 aa, Homo sapiens
ASTKGPSVFPLAPCSRSTSESTAALGCLVKDYFPEPVTVSWNSGALTSGVHTFPAVLQSSGLYSLSSVVTVPSSNFGTQTYTCNVDHKPSNTKVDKTVERKCCVECPPCPAPPVAGPSVFLFPPKPKDTLMISRTPEVTCVVVDVSHEDPEVQFNWYVDGVEVHNAKTKPREEQFNSTFRVVSVLTVVHQDWLNGKEYKCKVSNKGLPAPIEKTISKTKGQPREPQVYTLPPSREEMTKNQVSLTCLVKGFYPSDISVEWESNGQPENNYKTTPPMLDSDGSFFLYSKLTVDKSRWQQGNVFSCSVMHEALHNHYTQKSLSLSPGK

SEQ ID NO: 49 - protein, 377 aa, Homo sapiens
ASTKGPSVFPLAPCSRSTSGGTAALGCLVKDYFPEPVTVSWNSGALTSGVHTFPAVLQSSGLYSLSSVVTVPSSSLGTQTYTCNVNHKPSNTKVDKRVELKTPLGDTTHTCPRCPEPKSCDTPPPCPRCPEPKSCDTPPPCPRCPEPKSCDTPPPCPRCPAPELLGGPSVFLFPPKPKDTLMISRTPEVTCVVVDVSHEDPEVQFKWYVDGVEVHNAKTKPREEQYNSTFRVVSVLTVLHQDWLNGKEYKCKVSNKALPAPIEKTISKTKGQPREPQVYTLPPSREEMTKNQVSLTCLVKGFYPSDIAVEWESSGQPENNYNTTPPMLDSDGSFFLYSKLTVDKSRWQQGNIFSCSVMHEALHNRFTQKSLSLSPGK

SEQ ID NO: 50 - protein, 327 aa, Homo sapiens
ASTKGPSVFPLAPCSRSTSESTAALGCLVKDYFPEPVTVSWNSGALTSGVHTFPAVLQSSGLYSLSSVVTVPSSSLGTKTYTCNVDHKPSNTKVDKRVESKYGPPCPSCPAPEFLGGPSVFLFPPKPKDTLMISRTPEVTCVVVDVSQEDPEVQFNWYVDGVEVHNAKTKPREEQFNSTYRVVSVLTVLHQDWLNGKEYKCKVSNKGLPSSIEKTISKAKGQPREPQVYTLPPSQEEMTKNQVSLTCLVKGFYPSDIAVEWESNGQPENNYKTTPPVLDSDGSFFLYSRLTVDKSRWQEGNVFSCSVMHEALHNHYTQKSLSLSLGK

SEQ ID NO: 51 - protein, 453 aa, Homo sapiens
GSASAPTLFPLVSCENSPSDTSSVAVGCLAQDFLPDSITFSWKYKNNSDISSTRGFPSVLRGGKYAATSQVLLPSKDVMQGTDEHVVCKVQHPNGNKEKNVPLPVIAELPPKVSVFVPPRDGFFGNPRKSKLICQATGFSPRQIQVSWLREGKQVGSGVTTDQVQAEAKESGPTTYKVTSTLTIKESDWLGQSMFTCRVDHRGLTFQQNASSMCVPDQDTAIRVFAIPPSFASIFLTKSTKLTCLVTDLTTYDSVTISWTRQNGEAVKTHTNISESHPNATFSAVGEASICEDDWNSGERFTCTVTHTDLPSPLKQTISRPKGVALHRPDVYLLPPAREQLNLRESATITCLVTGFSPADVFVQWMQRGQPLSPEKYVTSAPMPEPQAPGRYFAHSILTVSEEEWNTGETYTCVVAHEALPNRVTERTVDKSTGKPTLYNVSLVMSDTAGTCY

SEQ ID NO: 52 - protein, 106 aa, Homo sapiens
GQPKANPTVTLFPPSSEELQANKATLVCLISDFYPGAVTVAWKADGSPVKAGVETTKPSKQSNNKYAASSYLSLTPEQWKSHRSYSCQVTHEGSTVEKTVAPTECS

SEQ ID NO: 53 - protein, 106 aa, Homo sp.
GQPKAAPSVTLFPPSSEELQANKATLVCLISDFYPGAVTVAWKADSSPVKAGVETTTPSKQSNNKYAASSYLSLTPEQWKSHRSYSCQVTHEGSTVEKTVAPTECS

SEQ ID NO: 54 - protein, 106 aa, Homo sapiens
GQPKAAPSVTLFPPSSEELQANKATLVCLISDFYPGAVTVAWKADSSPVKAGVETTTPSKQSNNKYAASSYLSLTPEQWKSHKSYSCQVTHEGSTVEKTVAPTECS

SEQ ID NO: 55 - protein, 106 aa, Homo sapiens
GQPKAAPSVTLFPPSSEELQANKATLVCLISDFYPGAVKVAWKADGSPVNTGVETTTPSKQSNNKYAASSYLSLTPEQWKSHRSYSCQVTHEGSTVEKTVAPAECS

SEQ ID NO: 56 - protein, 106 aa, Homo sapiens
GQPKAAPSVTLFPPSSEELQANKATLVCLVSDFNPGAVTVAWKADGSPVKVGVETTKPSKQSNNKYAASSYLSLTPEQWKSHRSYSCRVTHEGSTVEKTVAPAECS

SEQ ID NO: 57 - protein, 107 aa, Homo sapiens [sequence omitted]